European Patent Application EP 4 273 228 A1, published November 8, 2023. Title: Strain Having Enhanced L-Glutamic Acid Production Capacity,and Method for Construction the Same and Use Thereof. Applicant: NINGXIA EPPEN BIOTECH CO., LTD. The sequence listing filed with the application follows.

SEQUENCE LISTING (49 sequences)

SEQ ID NO: 1 - DNA, 1473 bp, Corynebacterium glutamicum
atgactattaatgtctccgaactacttgccaaagtccccacgggtctactgattggtgattcctgggtggaagcatccgagggcggtactttcgatgtggaaaacccagcgacgggtgaaacaatcgcaacgctcgcgtctgctacttccgaggatgcactggctgctcttgatgctgcatgcgctgttcaggccgagtgggctaggacgccagcgcgcgagcgttctaatattttacgacgcggtttcgagctcgtcgcggaacgtgcagaagagttcgccaccctcatgaccttggaaatgggcaaacctttggctgaagctcgcggcgaagtcacctacggcaacgaattcctgcgctggttctctgaggaagcagtccgcctctacggccgctacggtgctaccccagaaggcaacctgcgcatgatgaccacccgcaaaccagttggcccctgcctgttgatcaccccatggaacttcccactagcaatggccacccgtaaggttgcacccgccatcgctgcaggttgtgtcatggtgctcaagccagctcgcctgaccccgctgacctcccagtattttgcccagaccatgcttgatgccggtcttccagcaggtgtcctcaatgtggtctccggtgcttccgcctctgcgatttccaacccgattatggaagacgatcgccttcgtaaagtctcattcaccggctccaccccagttggccagcagctgctcaaaaaggctgccgataaagttctgcgcacctccatggaactcggcggcaacgcacctttcattgtcttcgaggacgccgacctagatctcgcgatcgaaggtgccatgggcgcaaaaatgcgcaacatcggcgaagcttgcaccgcagccaaccgtttcctagtccacgaatccgtcgccgatgaattcggccgacgcttcgcagcccgcctcgaggaacaagtcctaggcaacggcctcgacgaaggcgtcaccgtaggcccattggttgaggaaaaagcacgaaacagcgttgcatcgcttgtcgacgccgccgtctccgaaggtgccaccgtcctcaccggtggcaaggccggcacaggtgcaggctacttctacgaaccaacggtgctcacgggagtttcaacagatgcagccatcctgaacgaagagatcttcggtcccgtcgcaccgatcgtcaccttctctgatgaagctgaagctctgcgcctagccaattccaccgaatacggcctggcctcctacgtgttcacccaagacacctcacgcatcttccgcgtctccgacggcctcgagttcggcctagtgggcgtcaactccggtgtcatctctaacgccgctgcaccttttggtggcgtaaaacaatccggaatgggccgcgaaggtggtctcgaaggaattgaagagtacacctccgtgcagtacatcggtatccgggatccttacgccggctag

SEQ ID NO: 2 - DNA, 1473 bp, Corynebacterium glutamicum
atgactattaatgtctccgaactacttgccaaagtccccacgggtctactgattggtgattcctgggtggaagcatccgagggcggtactttcgatgtggaaaacccagcgacgggtgaaacaatcgcaacgctcgcgtctgctacttccgaggatgcactggctgctcttgatgctgcatgcgctgttcaggccgagtgggctaggacgccagcgcgcgagcgttctaatattttacgacgcggtttcgagctcgtcgcggaacgtgcagaagagttcgccaccctcatgaccttggaaatgggcaaacctttggctgaagctcgcggcgaagtcacctacggcaacgaattcctgcgctggttctctgaggaagcagtccgcctctacggccgctacggtgctaccccagaaggcaacctgcgcatgatgaccacccgcaaaccagttggcccctgcctgttgatcaccccatggaacttcccactagcaatggccacccgtaaggttgcacccgccatcgctgcaggttgtgtcatggtgctcaagccagctcgcctgaccccgctgacctcccagtattttgcccagaccatacttgatgccggtcttccagcaggtgtcctcaatgtggtctccggtgcttccgcctctgcgatttccaacccgattatggaagacgatcgccttcgtaaagtctcattcaccggctccaccccagttggccagcagctgctcaaaaaggctgccgataaagttctgcgcacctccatggaactcggcggcaacgcacctttcattgtcttcgaggacgccgacctagatctcgcgatcgaaggtgccatgggcgcaaaaatgcgcaacatcggcgaagcttgcaccgcagccaaccgtttcctagtccacgaatccgtcgccgatgaattcggccgacgcttcgcagcccgcctcgaggaacaagtcctaggcaacggcctcgacgaaggcgtcaccgtaggcccattggttgaggaaaaagcacgaaacagcgttgcatcgcttgtcgacgccgccgtctccgaaggtgccaccgtcctcaccggtggcaaggccggcacaggtgcaggctacttctacgaaccaacggtgctcacgggagtttcaacagatgcagccatcctgaacgaagagatcttcggtcccgtcgcaccgatcgtcaccttctctgatgaagctgaagctctgcgcctagccaattccaccgaatacggcctggcctcctacgtgttcacccaagacacctcacgcatcttccgcgtctccgacggcctcgagttcggcctagtgggcgtcaactccggtgtcatctctaacgccgctgcaccttttggtggcgtaaaacaatccggaatgggccgcgaaggtggtctcgaaggaattgaagagtacacctccgtgcagtacatcggtatccgggatccttacgccggctag

SEQ ID NO: 3 - protein, 490 aa, Corynebacterium glutamicum
MTINVSELLAKVPTGLLIGDSWVEASEGGTFDVENPATGETIATLASATSEDALAALDAACAVQAEWARTPARERSNILRRGFELVAERAEEFATLMTLEMGKPLAEARGEVTYGNEFLRWFSEEAVRLYGRYGATPEGNLRMMTTRKPVGPCLLITPWNFPLAMATRKVAPAIAAGCVMVLKPARLTPLTSQYFAQTMLDAGLPAGVLNVVSGASASAISNPIMEDDRLRKVSFTGSTPVGQQLLKKAADKVLRTSMELGGNAPFIVFEDADLDLAIEGAMGAKMRNIGEACTAANRFLVHESVADEFGRRFAARLEEQVLGNGLDEGVTVGPLVEEKARNSVASLVDAAVSEGATVLTGGKAGTGAGYFYEPTVLTGVSTDAAILNEEIFGPVAPIVTFSDEAEALRLANSTEYGLASYVFTQDTSRIFRVSDGLEFGLVGVNSGVISNAAAPFGGVKQSGMGREGGLEGIEEYTSVQYIGIRDPYAG

SEQ ID NO: 4 - protein, 490 aa, Corynebacterium glutamicum
MTINVSELLAKVPTGLLIGDSWVEASEGGTFDVENPATGETIATLASATSEDALAALDAACAVQAEWARTPARERSNILRRGFELVAERAEEFATLMTLEMGKPLAEARGEVTYGNEFLRWFSEEAVRLYGRYGATPEGNLRMMTTRKPVGPCLLITPWNFPLAMATRKVAPAIAAGCVMVLKPARLTPLTSQYFAQTILDAGLPAGVLNVVSGASASAISNPIMEDDRLRKVSFTGSTPVGQQLLKKAADKVLRTSMELGGNAPFIVFEDADLDLAIEGAMGAKMRNIGEACTAANRFLVHESVADEFGRRFAARLEEQVLGNGLDEGVTVGPLVEEKARNSVASLVDAAVSEGATVLTGGKAGTGAGYFYEPTVLTGVSTDAAILNEEIFGPVAPIVTFSDEAEALRLANSTEYGLASYVFTQDTSRIFRVSDGLEFGLVGVNSGVISNAAAPFGGVKQSGMGREGGLEGIEEYTSVQYIGIRDPYAG

SEQ ID NO: 5 - DNA, 56 bp, Artificial Sequence
  Synthesized
cagtgccaagcttgcatgcctgcaggtcgactctagatgactattaatgtctccga

SEQ ID NO: 6 - DNA, 27 bp, Artificial Sequence
  Synthesized
agaccggcatcaagtatggtctgggca

SEQ ID NO: 7 - DNA, 27 bp, Artificial Sequence
  Synthesized
tgcccagaccatacttgatgccggtct

SEQ ID NO: 8 - DNA, 62 bp, Artificial Sequence
  Synthesized
cagctatgaccatgattacgaattcgagctcggtacccctagccggcgtaaggatcccggat

SEQ ID NO: 9 - DNA, 20 bp, Artificial Sequence
  Synthesized
agaaggcaacctgcgcatga

SEQ ID NO: 10 - DNA, 20 bp, Artificial Sequence
  Synthesized
atcgggttggaaatcgcaga

SEQ ID NO: 11 - DNA, 56 bp, Artificial Sequence
  Synthesized
cagtgccaagcttgcatgcctgcaggtcgactctaggacccgcttgccatacgaag

SEQ ID NO: 12 - DNA, 40 bp, Artificial Sequence
  Synthesized
cctaccacgacgagcactacatctactcatctgaagaatc

SEQ ID NO: 13 - DNA, 40 bp, Artificial Sequence
  Synthesized
gattcttcagatgagtagatgtagtgctcgtcgtggtagg

SEQ ID NO: 14 - DNA, 40 bp, Artificial Sequence
  Synthesized
caaaccagagtgcccacgaactagccggcgtaaggatccc

SEQ ID NO: 15 - DNA, 40 bp, Artificial Sequence
  Synthesized
gggatccttacgccggctagttcgtgggcactctggtttg

SEQ ID NO: 16 - DNA, 58 bp, Artificial Sequence
  Synthesized
cagctatgaccatgattacgaattcgagctcggtaccccataagaaacaaccacttcc

SEQ ID NO: 17 - DNA, 20 bp, Artificial Sequence
  Synthesized
gtccaaggtgacggccgcac

SEQ ID NO: 18 - DNA, 20 bp, Artificial Sequence
  Synthesized
agcttcgccgatgttgcgca

SEQ ID NO: 19 - DNA, 23 bp, Artificial Sequence
  Synthesized
aggttgcacccgccatcgctgca

SEQ ID NO: 20 - DNA, 20 bp, Artificial Sequence
  Synthesized
atattcggcccagcagcagc

SEQ ID NO: 21 - DNA, 56 bp, Artificial Sequence
  Synthesized
gcttgcatgcctgcaggtcgactctagaggatccccgtagtgctcgtcgtggtagg

SEQ ID NO: 22 - DNA, 58 bp, Artificial Sequence
  Synthesized
atcaggctgaaaatcttctctcatccgccaaaacctagccggcgtaaggatcccggat

SEQ ID NO: 23 - DNA, 56 bp, Artificial Sequence
  Synthesized
cagtgccaagcttgcatgcctgcaggtcgactctaggtctgggggtgagcgcggat

SEQ ID NO: 24 - DNA, 54 bp, Artificial Sequence
  Synthesized
aggaaaataacgcatccatctgcccctttacaaatccaccgcaaacactgggat

SEQ ID NO: 25 - DNA, 54 bp, Artificial Sequence
  Synthesized
tggatttgtaaaggggcagatggatgcgttattttccttcacttttcgtatcca

SEQ ID NO: 26 - DNA, 65 bp, Artificial Sequence
  Synthesized
cagctatgaccatgattacgaattcgagctcggtacccctctggcgcatcgaacaggtcgaagga

SEQ ID NO: 27 - DNA, 20 bp, Artificial Sequence
  Synthesized
gtctgggggtgagcgcggat

SEQ ID NO: 28 - DNA, 27 bp, Artificial Sequence
  Synthesized
ctctggcgcatcgaacaggtcgaagga

SEQ ID NO: 29 - DNA, 647 bp, Artificial Sequence
  Synthesized
cagtgccaagcttgcatgcctgcaggtcgactctagatgactattaatgtctccgaactacttgccaaagtccccacgggtctactgattggtgattcctgggtggaagcatccgagggcggtactttcgatgtggaaaacccagcgacgggtgaaacaatcgcaacgctcgcgtctgctacttccgaggatgcactggctgctcttgatgctgcatgcgctgttcaggccgagtgggctaggacgccagcgcgcgagcgttctaatattttacgacgcggtttcgagctcgtcgcggaacgtgcagaagagttcgccaccctcatgaccttggaaatgggcaaacctttggctgaagctcgcggcgaagtcacctacggcaacgaattcctgcgctggttctctgaggaagcagtccgcctctacggccgctacggtgctaccccagaaggcaacctgcgcatgatgaccacccgcaaaccagttggcccctgcctgttgatcaccccatggaacttcccactagcaatggccacccgtaaggttgcacccgccatcgctgcaggttgtgtcatggtgctcaagccagctcgcctgaccccgctgacctcccagtattttgcccagaccatacttgatgccggtct

SEQ ID NO: 30 - DNA, 927 bp, Artificial Sequence
  Synthesized
tgcccagaccatacttgatgccggtcttccagcaggtgtcctcaatgtggtctccggtgcttccgcctctgcgatttccaacccgattatggaagacgatcgccttcgtaaagtctcattcaccggctccaccccagttggccagcagctgctcaaaaaggctgccgataaagttctgcgcacctccatggaactcggcggcaacgcacctttcattgtcttcgaggacgccgacctagatctcgcgatcgaaggtgccatgggcgcaaaaatgcgcaacatcggcgaagcttgcaccgcagccaaccgtttcctagtccacgaatccgtcgccgatgaattcggccgacgcttcgcagcccgcctcgaggaacaagtcctaggcaacggcctcgacgaaggcgtcaccgtaggcccattggttgaggaaaaagcacgaaacagcgttgcatcgcttgtcgacgccgccgtctccgaaggtgccaccgtcctcaccggtggcaaggccggcacaggtgcaggctacttctacgaaccaacggtgctcacgggagtttcaacagatgcagccatcctgaacgaagagatcttcggtcccgtcgcaccgatcgtcaccttctctgatgaagctgaagctctgcgcctagccaattccaccgaatacggcctggcctcctacgtgttcacccaagacacctcacgcatcttccgcgtctccgacggcctcgagttcggcctagtgggcgtcaactccggtgtcatctctaacgccgctgcaccttttggtggcgtaaaacaatccggaatgggccgcgaaggtggtctcgaaggaattgaagagtacacctccgtgcagtacatcggtatccgggatccttacgccggctaggggtaccgagctcgaattcgtaatcatggtcatagctg

SEQ ID NO: 31 - DNA, 1547 bp, Artificial Sequence
  Synthesized
cagtgccaagcttgcatgcctgcaggtcgactctagatgactattaatgtctccgaactacttgccaaagtccccacgggtctactgattggtgattcctgggtggaagcatccgagggcggtactttcgatgtggaaaacccagcgacgggtgaaacaatcgcaacgctcgcgtctgctacttccgaggatgcactggctgctcttgatgctgcatgcgctgttcaggccgagtgggctaggacgccagcgcgcgagcgttctaatattttacgacgcggtttcgagctcgtcgcggaacgtgcagaagagttcgccaccctcatgaccttggaaatgggcaaacctttggctgaagctcgcggcgaagtcacctacggcaacgaattcctgcgctggttctctgaggaagcagtccgcctctacggccgctacggtgctaccccagaaggcaacctgcgcatgatgaccacccgcaaaccagttggcccctgcctgttgatcaccccatggaacttcccactagcaatggccacccgtaaggttgcacccgccatcgctgcaggttgtgtcatggtgctcaagccagctcgcctgaccccgctgacctcccagtattttgcccagaccatacttgatgccggtcttccagcaggtgtcctcaatgtggtctccggtgcttccgcctctgcgatttccaacccgattatggaagacgatcgccttcgtaaagtctcattcaccggctccaccccagttggccagcagctgctcaaaaaggctgccgataaagttctgcgcacctccatggaactcggcggcaacgcacctttcattgtcttcgaggacgccgacctagatctcgcgatcgaaggtgccatgggcgcaaaaatgcgcaacatcggcgaagcttgcaccgcagccaaccgtttcctagtccacgaatccgtcgccgatgaattcggccgacgcttcgcagcccgcctcgaggaacaagtcctaggcaacggcctcgacgaaggcgtcaccgtaggcccattggttgaggaaaaagcacgaaacagcgttgcatcgcttgtcgacgccgccgtctccgaaggtgccaccgtcctcaccggtggcaaggccggcacaggtgcaggctacttctacgaaccaacggtgctcacgggagtttcaacagatgcagccatcctgaacgaagagatcttcggtcccgtcgcaccgatcgtcaccttctctgatgaagctgaagctctgcgcctagccaattccaccgaatacggcctggcctcctacgtgttcacccaagacacctcacgcatcttccgcgtctccgacggcctcgagttcggcctagtgggcgtcaactccggtgtcatctctaacgccgctgcaccttttggtggcgtaaaacaatccggaatgggccgcgaaggtggtctcgaaggaattgaagagtacacctccgtgcagtacatcggtatccgggatccttacgccggctaggggtaccgagctcgaattcgtaatcatggtcatagctg

SEQ ID NO: 32 - DNA, 1554 bp, Artificial Sequence
  Synthesized
cagtgccaagcttgcatgcctgcaggtcgactctagatgactattaatgtctccgaactacttgccaaagtccccacgggtctactgattggtgattcctgggtggaagcatccgagggcggtactttcgatgtggaaaacccagcgacgggtgaaacaatcgcaacgctcgcgtctgctacttccgaggatgcactggctgctcttgatgctgcatgcgctgttcaggccgagtgggctaggacgccagcgcgcgagcgttctaatattttacgacgcggtttcgagctcgtcgcggaacgtgcagaagagttcgccaccctcatgaccttggaaatgggcaaacctttggctgaagctcgcggcgaagtcacctacggcaacgaattcctgcgctggttctctgaggaagcagtccgcctctacggccgctacggtgctaccccagaaggcaacctgcgcatgatgaccacccgcaaaccagttggcccctgcctgttgatcaccccatggaacttcccactagcaatggccacccgtaaggttgcacccgccatcgctgcaggttgtgtcatggtgctcaagccagctcgcctgaccccgctgacctcccagtattttgcccagaccatacttgatgccggtcttccagcaggtgtcctcaatgtggtctccggtgcttccgcctctgcgatttccaacccgattatggaagacgatcgccttcgtaaagtctcattcaccggctccaccccagttggccagcagctgctcaaaaaggctgccgataaagttctgcgcacctccatggaactcggcggcaacgcacctttcattgtcttcgaggacgccgacctagatctcgcgatcgaaggtgccatgggcgcaaaaatgcgcaacatcggcgaagcttgcaccgcagccaaccgtttcctagtccacgaatccgtcgccgatgaattcggccgacgcttcgcagcccgcctcgaggaacaagtcctaggcaacggcctcgacgaaggcgtcaccgtaggcccattggttgaggaaaaagcacgaaacagcgttgcatcgcttgtcgacgccgccgtctccgaaggtgccaccgtcctcaccggtggcaaggccggcacaggtgcaggctacttctacgaaccaacggtgctcacgggagtttcaacagatgcagccatcctgaacgaagagatcttcggtcccgtcgcaccgatcgtcaccttctctgatgaagctgaagctctgcgcctagccaattccaccgaatacggcctggcctcctacgtgttcacccaagacacctcacgcatcttccgcgtctccgacggcctcgagttcggcctagtgggcgtcaactccggtgtcatctctaacgccgctgcaccttttggtggcgtaaaacaatccggaatgggccgcgaaggtggtctcgaaggaattgaagagtacacctccgtgcagtacatcggtatccgggatccttacgccggctaggggtaccgagctcgaattcgtaatcatggtcatagctgtttcctg

SEQ ID NO: 33 - DNA, 261 bp, Artificial Sequence
  Synthesized
agaaggcaacctgcgcatgatgaccacccgcaaaccagttggcccctgcctgttgatcaccccatggaacttcccactagcaatggccacccgtaaggttgcacccgccatcgctgcaggttgtgtcatggtgctcaagccagctcgcctgaccccgctgacctcccagtattttgcccagaccatgcttgatgccggtcttccagcaggtgtcctcaatgtggtctccggtgcttccgcctctgcgatttccaacccgat

SEQ ID NO: 34 - DNA, 806 bp, Artificial Sequence
  Synthesized
cagtgccaagcttgcatgcctgcaggtcgactctaggacccgcttgccatacgaagtcctggagaagatctccacccgcatcaccaacgaagttccagacgtaaaccgcgtggttttggacgtaacctccaagccaccaggaaccatcgaatgggagtaggccttaaatgagccttcgttaagcggcaatcaccttatcggtgattgccgctttcccatttctccgggttttctggaactttttgggcgtatgctgggaatgatcttattattttgatttcagaaagcaggagagaccagatgagcgaaatccttgaaacctactgggcaccccacttcggaaacaccgatgaagccgcagcactcgtttcatacttggcacaagcttccggtgatcctattgaggttcacaccctgttcggggatttaggtttagacggactctctggaaactacaccgacactgagatcgacggctacggcgacgcattcctgctggttgcagcactagcagtgttgatggctgaaaacaaagcatccggcggcgtgaatctgggtgaagttgggggagctgataaatcgatccggctgcatgttgaatccaaggaaaacacccagatcaacaccgcattgaagtactttgcgctttccccagaagaccacgcagcggcagatcgcttcgatgaggatgacctgtctgagcttgccaacttgagtgaagagctgcgcggacagctggactaattgctgcccgtttaaggagtccgattcttcagatgagtagatgtagtgctcgtcgtggtagg

SEQ ID NO: 35 - DNA, 1777 bp, Artificial Sequence
  Synthesized
gattcttcagatgagtagatgtagtgctcgtcgtggtaggtgcgcagcagagattcaggcgcacgaccagaaagcacgtggctgagcttccagccggacgttgtggccggagtaaaaatccatccaaactttccgcgatgctggtaaacctgtggatgtcaatgcctttgatttgaactaagcacaggactacctcgacgccggcgccaactttgtccgagtcggtgccgatgtccagcaactcaacgctgctggatacgaaaagtgaaggaaaataacgcatcatgactattaatgtctccgaactacttgccaaagtccccacgggtctactgattggtgattcctgggtggaagcatccgagggcggtactttcgatgtggaaaacccagcgacgggtgaaacaatcgcaacgctcgcgtctgctacttccgaggatgcactggctgctcttgatgctgcatgcgctgttcaggccgagtgggctaggacgccagcgcgcgagcgttctaatattttacgacgcggtttcgagctcgtcgcggaacgtgcagaagagttcgccaccctcatgaccttggaaatgggcaaacctttggctgaagctcgcggcgaagtcacctacggcaacgaattcctgcgctggttctctgaggaagcagtccgcctctacggccgctacggtgctaccccagaaggcaacctgcgcatgatgaccacccgcaaaccagttggcccctgcctgttgatcaccccatggaacttcccactagcaatggccacccgtaaggttgcacccgccatcgctgcaggttgtgtcatggtgctcaagccagctcgcctgaccccgctgacctcccagtattttgcccagaccatgcttgatgccggtcttccagcaggtgtcctcaatgtggtctccggtgcttccgcctctgcgatttccaacccgattatggaagacgatcgccttcgtaaagtctcattcaccggctccaccccagttggccagcagctgctcaaaaaggctgccgataaagttctgcgcacctccatggaactcggcggcaacgcacctttcattgtcttcgaggacgccgacctagatctcgcgatcgaaggtgccatgggcgcaaaaatgcgcaacatcggcgaagcttgcaccgcagccaaccgtttcctagtccacgaatccgtcgccgatgaattcggccgacgcttcgcagcccgcctcgaggaacaagtcctaggcaacggcctcgacgaaggcgtcaccgtaggcccattggttgaggaaaaagcacgaaacagcgttgcatcgcttgtcgacgccgccgtctccgaaggtgccaccgtcctcaccggtggcaaggccggcacaggtgcaggctacttctacgaaccaacggtgctcacgggagtttcaacagatgcagccatcctgaacgaagagatcttcggtcccgtcgcaccgatcgtcaccttctctgatgaagctgaagctctgcgcctagccaattccaccgaatacggcctggcctcctacgtgttcacccaagacacctcacgcatcttccgcgtctccgacggcctcgagttcggcctagtgggcgtcaactccggtgtcatctctaacgccgctgcaccttttggtggcgtaaaacaatccggaatgggccgcgaaggtggtctcgaaggaattgaagagtacacctccgtgcagtacatcggtatccgggatccttacgccggctagttcgtgggcactctggtttg

SEQ ID NO: 36 - DNA, 1777 bp, Artificial Sequence
  Synthesized
gattcttcagatgagtagatgtagtgctcgtcgtggtaggtgcgcagcagagattcaggcgcacgaccagaaagcacgtggctgagcttccagccggacgttgtggccggagtaaaaatccatccaaactttccgcgatgctggtaaacctgtggatgtcaatgcctttgatttgaactaagcacaggactacctcgacgccggcgccaactttgtccgagtcggtgccgatgtccagcaactcaacgctgctggatacgaaaagtgaaggaaaataacgcatcatgactattaatgtctccgaactacttgccaaagtccccacgggtctactgattggtgattcctgggtggaagcatccgagggcggtactttcgatgtggaaaacccagcgacgggtgaaacaatcgcaacgctcgcgtctgctacttccgaggatgcactggctgctcttgatgctgcatgcgctgttcaggccgagtgggctaggacgccagcgcgcgagcgttctaatattttacgacgcggtttcgagctcgtcgcggaacgtgcagaagagttcgccaccctcatgaccttggaaatgggcaaacctttggctgaagctcgcggcgaagtcacctacggcaacgaattcctgcgctggttctctgaggaagcagtccgcctctacggccgctacggtgctaccccagaaggcaacctgcgcatgatgaccacccgcaaaccagttggcccctgcctgttgatcaccccatggaacttcccactagcaatggccacccgtaaggttgcacccgccatcgctgcaggttgtgtcatggtgctcaagccagctcgcctgaccccgctgacctcccagtattttgcccagaccatacttgatgccggtcttccagcaggtgtcctcaatgtggtctccggtgcttccgcctctgcgatttccaacccgattatggaagacgatcgccttcgtaaagtctcattcaccggctccaccccagttggccagcagctgctcaaaaaggctgccgataaagttctgcgcacctccatggaactcggcggcaacgcacctttcattgtcttcgaggacgccgacctagatctcgcgatcgaaggtgccatgggcgcaaaaatgcgcaacatcggcgaagcttgcaccgcagccaaccgtttcctagtccacgaatccgtcgccgatgaattcggccgacgcttcgcagcccgcctcgaggaacaagtcctaggcaacggcctcgacgaaggcgtcaccgtaggcccattggttgaggaaaaagcacgaaacagcgttgcatcgcttgtcgacgccgccgtctccgaaggtgccaccgtcctcaccggtggcaaggccggcacaggtgcaggctacttctacgaaccaacggtgctcacgggagtttcaacagatgcagccatcctgaacgaagagatcttcggtcccgtcgcaccgatcgtcaccttctctgatgaagctgaagctctgcgcctagccaattccaccgaatacggcctggcctcctacgtgttcacccaagacacctcacgcatcttccgcgtctccgacggcctcgagttcggcctagtgggcgtcaactccggtgtcatctctaacgccgctgcaccttttggtggcgtaaaacaatccggaatgggccgcgaaggtggtctcgaaggaattgaagagtacacctccgtgcagtacatcggtatccgggatccttacgccggctagttcgtgggcactctggtttg

SEQ ID NO: 37 - DNA, 788 bp, Artificial Sequence
  Synthesized
gggatccttacgccggctagttcgtgggcactctggtttggttaccaggatgggttagtcattctgatcagcgaattccacgttcacatcgccaattccagagttcacaaccagattcagcattggaccttctagatcagcattgtgggcggtgagatctccaacatcacagcgcgctgtgcccacaccggcggtacaacttaggctcacgggcacatcatcgggcagggtgaccatgacttcgccgatccctgaggtgatttggatgttttgttcctgatccaattgggtgaggtggctgaaatcgaggttcatttcacccacgccagaggtgtagctgctgaggagttcatcgttggtggggatgagattgacatcgccgattccagggtcgtcttcaaagtagatgggatcgatatttgaaataaacaggcctgcgagggcgctcatgacaactccggtaccaactacaccgccgacaatccatggccacacatggcgctttttctgaggcttttgtggagggacttgtacatcccaggtgttgtattggttttgggcaagtggatcccaatgaggcgcttcgggggtttgttgcgcgaagggtgcatagtagccctcaacgggggtgatagtgcttagatctggttggggttgtgggtagagatcttcgtttttcatggtggcatcctcagaaacagtgaattcagtggtgagtagtccgcggggtggaagtggttgtttcttatggggtaccgagctcgaattcgtaatcatggtcatagctg

SEQ ID NO: 38 - DNA, 3291 bp, Artificial Sequence
  Synthesized
cagtgccaagcttgcatgcctgcaggtcgactctaggacccgcttgccatacgaagtcctggagaagatctccacccgcatcaccaacgaagttccagacgtaaaccgcgtggttttggacgtaacctccaagccaccaggaaccatcgaatgggagtaggccttaaatgagccttcgttaagcggcaatcaccttatcggtgattgccgctttcccatttctccgggttttctggaactttttgggcgtatgctgggaatgatcttattattttgatttcagaaagcaggagagaccagatgagcgaaatccttgaaacctactgggcaccccacttcggaaacaccgatgaagccgcagcactcgtttcatacttggcacaagcttccggtgatcctattgaggttcacaccctgttcggggatttaggtttagacggactctctggaaactacaccgacactgagatcgacggctacggcgacgcattcctgctggttgcagcactagcagtgttgatggctgaaaacaaagcatccggcggcgtgaatctgggtgaagttgggggagctgataaatcgatccggctgcatgttgaatccaaggaaaacacccagatcaacaccgcattgaagtactttgcgctttccccagaagaccacgcagcggcagatcgcttcgatgaggatgacctgtctgagcttgccaacttgagtgaagagctgcgcggacagctggactaattgctgcccgtttaaggagtccgattcttcagatgagtagatgtagtgctcgtcgtggtaggtgcgcagcagagattcaggcgcacgaccagaaagcacgtggctgagcttccagccggacgttgtggccggagtaaaaatccatccaaactttccgcgatgctggtaaacctgtggatgtcaatgcctttgatttgaactaagcacaggactacctcgacgccggcgccaactttgtccgagtcggtgccgatgtccagcaactcaacgctgctggatacgaaaagtgaaggaaaataacgcatcatgactattaatgtctccgaactacttgccaaagtccccacgggtctactgattggtgattcctgggtggaagcatccgagggcggtactttcgatgtggaaaacccagcgacgggtgaaacaatcgcaacgctcgcgtctgctacttccgaggatgcactggctgctcttgatgctgcatgcgctgttcaggccgagtgggctaggacgccagcgcgcgagcgttctaatattttacgacgcggtttcgagctcgtcgcggaacgtgcagaagagttcgccaccctcatgaccttggaaatgggcaaacctttggctgaagctcgcggcgaagtcacctacggcaacgaattcctgcgctggttctctgaggaagcagtccgcctctacggccgctacggtgctaccccagaaggcaacctgcgcatgatgaccacccgcaaaccagttggcccctgcctgttgatcaccccatggaacttcccactagcaatggccacccgtaaggttgcacccgccatcgctgcaggttgtgtcatggtgctcaagccagctcgcctgaccccgctgacctcccagtattttgcccagaccatgcttgatgccggtcttccagcaggtgtcctcaatgtggtctccggtgcttccgcctctgcgatttccaacccgattatggaagacgatcgccttcgtaaagtctcattcaccggctccaccccagttggccagcagctgctcaaaaaggctgccgataaagttctgcgcacctccatggaactcggcggcaacgcacctttcattgtcttcgaggacgccgacctagatctcgcgatcgaaggtgccatgggcgcaaaaatgcgcaacatcggcgaagcttgcaccgcagccaaccgtttcctagtccacgaatccgtcgccgatgaattcggccgacgcttcgcagcccgcctcgaggaacaagtcctaggcaacggcctcgacgaaggcgtcaccgtaggcccattggttgaggaaaaagcacgaaacagcgttgcatcgcttgtcgacgccgccgtctccgaaggtgccaccgtcctcaccggtggcaaggccggcacaggtgcaggctacttctacgaaccaacggtgctcacgggagtttcaacagatgcagccatcctgaacgaagagatcttcggtcccgtcgcaccgatcgtcaccttctctgatgaagctgaagctctgcgcctagccaattccaccgaatacggcctggcctcctacgtgttcacccaagacacctcacgcatcttccgcgtctccgacggcctcgagttcggcctagtgggcgtcaactccggtgtcatctctaacgccgctgcaccttttggtggcgtaaaacaatccggaatgggccgcgaaggtggtctcgaaggaattgaagagtacacctccgtgcagtacatcggtatccgggatccttacgccggctagttcgtgggcactctggtttggttaccaggatgggttagtcattctgatcagcgaattccacgttcacatcgccaattccagagttcacaaccagattcagcattggaccttctagatcagcattgtgggcggtgagatctccaacatcacagcgcgctgtgcccacaccggcggtacaacttaggctcacgggcacatcatcgggcagggtgaccatgacttcgccgatccctgaggtgatttggatgttttgttcctgatccaattgggtgaggtggctgaaatcgaggttcatttcacccacgccagaggtgtagctgctgaggagttcatcgttggtggggatgagattgacatcgccgattccagggtcgtcttcaaagtagatgggatcgatatttgaaataaacaggcctgcgagggcgctcatgacaactccggtaccaactacaccgccgacaatccatggccacacatggcgctttttctgaggcttttgtggagggacttgtacatcccaggtgttgtattggttttgggcaagtggatcccaatgaggcgcttcgggggtttgttgcgcgaagggtgcatagtagccctcaacgggggtgatagtgcttagatctggttggggttgtgggtagagatcttcgtttttcatggtggcatcctcagaaacagtgaattcagtggtgagtagtccgcggggtggaagtggttgtttcttatggggtaccgagctcgaattcgtaatcatggtcatagctg

SEQ ID NO: 39 - DNA, 3291 bp, Artificial Sequence
  Synthesized
cagtgccaagcttgcatgcctgcaggtcgactctaggacccgcttgccatacgaagtcctggagaagatctccacccgcatcaccaacgaagttccagacgtaaaccgcgtggttttggacgtaacctccaagccaccaggaaccatcgaatgggagtaggccttaaatgagccttcgttaagcggcaatcaccttatcggtgattgccgctttcccatttctccgggttttctggaactttttgggcgtatgctgggaatgatcttattattttgatttcagaaagcaggagagaccagatgagcgaaatccttgaaacctactgggcaccccacttcggaaacaccgatgaagccgcagcactcgtttcatacttggcacaagcttccggtgatcctattgaggttcacaccctgttcggggatttaggtttagacggactctctggaaactacaccgacactgagatcgacggctacggcgacgcattcctgctggttgcagcactagcagtgttgatggctgaaaacaaagcatccggcggcgtgaatctgggtgaagttgggggagctgataaatcgatccggctgcatgttgaatccaaggaaaacacccagatcaacaccgcattgaagtactttgcgctttccccagaagaccacgcagcggcagatcgcttcgatgaggatgacctgtctgagcttgccaacttgagtgaagagctgcgcggacagctggactaattgctgcccgtttaaggagtccgattcttcagatgagtagatgtagtgctcgtcgtggtaggtgcgcagcagagattcaggcgcacgaccagaaagcacgtggctgagcttccagccggacgttgtggccggagtaaaaatccatccaaactttccgcgatgctggtaaacctgtggatgtcaatgcctttgatttgaactaagcacaggactacctcgacgccggcgccaactttgtccgagtcggtgccgatgtccagcaactcaacgctgctggatacgaaaagtgaaggaaaataacgcatcatgactattaatgtctccgaactacttgccaaagtccccacgggtctactgattggtgattcctgggtggaagcatccgagggcggtactttcgatgtggaaaacccagcgacgggtgaaacaatcgcaacgctcgcgtctgctacttccgaggatgcactggctgctcttgatgctgcatgcgctgttcaggccgagtgggctaggacgccagcgcgcgagcgttctaatattttacgacgcggtttcgagctcgtcgcggaacgtgcagaagagttcgccaccctcatgaccttggaaatgggcaaacctttggctgaagctcgcggcgaagtcacctacggcaacgaattcctgcgctggttctctgaggaagcagtccgcctctacggccgctacggtgctaccccagaaggcaacctgcgcatgatgaccacccgcaaaccagttggcccctgcctgttgatcaccccatggaacttcccactagcaatggccacccgtaaggttgcacccgccatcgctgcaggttgtgtcatggtgctcaagccagctcgcctgaccccgctgacctcccagtattttgcccagaccatacttgatgccggtcttccagcaggtgtcctcaatgtggtctccggtgcttccgcctctgcgatttccaacccgattatggaagacgatcgccttcgtaaagtctcattcaccggctccaccccagttggccagcagctgctcaaaaaggctgccgataaagttctgcgcacctccatggaactcggcggcaacgcacctttcattgtcttcgaggacgccgacctagatctcgcgatcgaaggtgccatgggcgcaaaaatgcgcaacatcggcgaagcttgcaccgcagccaaccgtttcctagtccacgaatccgtcgccgatgaattcggccgacgcttcgcagcccgcctcgaggaacaagtcctaggcaacggcctcgacgaaggcgtcaccgtaggcccattggttgaggaaaaagcacgaaacagcgttgcatcgcttgtcgacgccgccgtctccgaaggtgccaccgtcctcaccggtggcaaggccggcacaggtgcaggctacttctacgaaccaacggtgctcacgggagtttcaacagatgcagccatcctgaacgaagagatcttcggtcccgtcgcaccgatcgtcaccttctctgatgaagctgaagctctgcgcctagccaattccaccgaatacggcctggcctcctacgtgttcacccaagacacctcacgcatcttccgcgtctccgacggcctcgagttcggcctagtgggcgtcaactccggtgtcatctctaacgccgctgcaccttttggtggcgtaaaacaatccggaatgggccgcgaaggtggtctcgaaggaattgaagagtacacctccgtgcagtacatcggtatccgggatccttacgccggctagttcgtgggcactctggtttggttaccaggatgggttagtcattctgatcagcgaattccacgttcacatcgccaattccagagttcacaaccagattcagcattggaccttctagatcagcattgtgggcggtgagatctccaacatcacagcgcgctgtgcccacaccggcggtacaacttaggctcacgggcacatcatcgggcagggtgaccatgacttcgccgatccctgaggtgatttggatgttttgttcctgatccaattgggtgaggtggctgaaatcgaggttcatttcacccacgccagaggtgtagctgctgaggagttcatcgttggtggggatgagattgacatcgccgattccagggtcgtcttcaaagtagatgggatcgatatttgaaataaacaggcctgcgagggcgctcatgacaactccggtaccaactacaccgccgacaatccatggccacacatggcgctttttctgaggcttttgtggagggacttgtacatcccaggtgttgtattggttttgggcaagtggatcccaatgaggcgcttcgggggtttgttgcgcgaagggtgcatagtagccctcaacgggggtgatagtgcttagatctggttggggttgtgggtagagatcttcgtttttcatggtggcatcctcagaaacagtgaattcagtggtgagtagtccgcggggtggaagtggttgtttcttatggggtaccgagctcgaattcgtaatcatggtcatagctg

SEQ ID NO: 40 - DNA, 1970 bp, Artificial Sequence
  Synthesized
gtccaaggtgacggccgcacctacggacacccaatcgtgctgcgcccagtatcttccgaagacgcaatgaccgccgactggacccgcttgccatacgaagtcctggagaagatctccacccgcatcaccaacgaagttccagacgtaaaccgcgtggttttggacgtaacctccaagccaccaggaaccatcgaatgggagtaggccttaaatgagccttcgttaagcggcaatcaccttatcggtgattgccgctttcccatttctccgggttttctggaactttttgggcgtatgctgggaatgatcttattattttgatttcagaaagcaggagagaccagatgagcgaaatccttgaaacctactgggcaccccacttcggaaacaccgatgaagccgcagcactcgtttcatacttggcacaagcttccggtgatcctattgaggttcacaccctgttcggggatttaggtttagacggactctctggaaactacaccgacactgagatcgacggctacggcgacgcattcctgctggttgcagcactagcagtgttgatggctgaaaacaaagcatccggcggcgtgaatctgggtgaagttgggggagctgataaatcgatccggctgcatgttgaatccaaggaaaacacccagatcaacaccgcattgaagtactttgcgctttccccagaagaccacgcagcggcagatcgcttcgatgaggatgacctgtctgagcttgccaacttgagtgaagagctgcgcggacagctggactaattgctgcccgtttaaggagtccgattcttcagatgagtagatgtagtgctcgtcgtggtaggtgcgcagcagagattcaggcgcacgaccagaaagcacgtggctgagcttccagccggacgttgtggccggagtaaaaatccatccaaactttccgcgatgctggtaaacctgtggatgtcaatgcctttgatttgaactaagcacaggactacctcgacgccggcgccaactttgtccgagtcggtgccgatgtccagcaactcaacgctgctggatacgaaaagtgaaggaaaataacgcatcatgactattaatgtctccgaactacttgccaaagtccccacgggtctactgattggtgattcctgggtggaagcatccgagggcggtactttcgatgtggaaaacccagcgacgggtgaaacaatcgcaacgctcgcgtctgctacttccgaggatgcactggctgctcttgatgctgcatgcgctgttcaggccgagtgggctaggacgccagcgcgcgagcgttctaatattttacgacgcggtttcgagctcgtcgcggaacgtgcagaagagttcgccaccctcatgaccttggaaatgggcaaacctttggctgaagctcgcggcgaagtcacctacggcaacgaattcctgcgctggttctctgaggaagcagtccgcctctacggccgctacggtgctaccccagaaggcaacctgcgcatgatgaccacccgcaaaccagttggcccctgcctgttgatcaccccatggaacttcccactagcaatggccacccgtaaggttgcacccgccatcgctgcaggttgtgtcatggtgctcaagccagctcgcctgaccccgctgacctcccagtattttgcccagaccatgcttgatgccggtcttccagcaggtgtcctcaatgtggtctccggtgcttccgcctctgcgatttccaacccgattatggaagacgatcgccttcgtaaagtctcattcaccggctccaccccagttggccagcagctgctcaaaaaggctgccgataaagttctgcgcacctccatggaactcggcggcaacgcacctttcattgtcttcgaggacgccgacctagatctcgcgatcgaaggtgccatgggcgcaaaaatgcgcaacatcggcgaagct

SEQ ID NO: 41 - DNA, 1758 bp, Artificial Sequence
  Synthesized
aggttgcacccgccatcgctgcaggttgtgtcatggtgctcaagccagctcgcctgaccccgctgacctcccagtattttgcccagaccatgcttgatgccggtcttccagcaggtgtcctcaatgtggtctccggtgcttccgcctctgcgatttccaacccgattatggaagacgatcgccttcgtaaagtctcattcaccggctccaccccagttggccagcagctgctcaaaaaggctgccgataaagttctgcgcacctccatggaactcggcggcaacgcacctttcattgtcttcgaggacgccgacctagatctcgcgatcgaaggtgccatgggcgcaaaaatgcgcaacatcggcgaagcttgcaccgcagccaaccgtttcctagtccacgaatccgtcgccgatgaattcggccgacgcttcgcagcccgcctcgaggaacaagtcctaggcaacggcctcgacgaaggcgtcaccgtaggcccattggttgaggaaaaagcacgaaacagcgttgcatcgcttgtcgacgccgccgtctccgaaggtgccaccgtcctcaccggtggcaaggccggcacaggtgcaggctacttctacgaaccaacggtgctcacgggagtttcaacagatgcagccatcctgaacgaagagatcttcggtcccgtcgcaccgatcgtcaccttctctgatgaagctgaagctctgcgcctagccaattccaccgaatacggcctggcctcctacgtgttcacccaagacacctcacgcatcttccgcgtctccgacggcctcgagttcggcctagtgggcgtcaactccggtgtcatctctaacgccgctgcaccttttggtggcgtaaaacaatccggaatgggccgcgaaggtggtctcgaaggaattgaagagtacacctccgtgcagtacatcggtatccgggatccttacgccggctagttcgtgggcactctggtttggttaccaggatgggttagtcattctgatcagcgaattccacgttcacatcgccaattccagagttcacaaccagattcagcattggaccttctagatcagcattgtgggcggtgagatctccaacatcacagcgcgctgtgcccacaccggcggtacaacttaggctcacgggcacatcatcgggcagggtgaccatgacttcgccgatccctgaggtgatttggatgttttgttcctgatccaattgggtgaggtggctgaaatcgaggttcatttcacccacgccagaggtgtagctgctgaggagttcatcgttggtggggatgagattgacatcgccgattccagggtcgtcttcaaagtagatgggatcgatatttgaaataaacaggcctgcgagggcgctcatgacaactccggtaccaactacaccgccgacaatccatggccacacatggcgctttttctgaggcttttgtggagggacttgtacatcccaggtgttgtattggttttgggcaagtggatcccaatgaggcgcttcgggggtttgttgcgcgaagggtgcatagtagccctcaacgggggtgatagtgcttagatctggttggggttgtgggtagagatcttcgtttttcatggtggcatcctcagaaacagtgaattcagtggtgagtagtccgcggggtggaagtggttgtttcttatgcaacgcccaccacatggctaaaaggcaaaggtaagtaatggctgctgctgggccgaatat

SEQ ID NO: 42 - DNA, 1807 bp, Artificial Sequence
  Synthesized
gcttgcatgcctgcaggtcgactctagaggatccccgtagtgctcgtcgtggtaggtgcgcagcagagattcaggcgcacgaccagaaagcacgtggctgagcttccagccggacgttgtggccggagtaaaaatccatccaaactttccgcgatgctggtaaacctgtggatgtcaatgcctttgatttgaactaagcacaggactacctcgacgccggcgccaactttgtccgagtcggtgccgatgtccagcaactcaacgctgctggatacgaaaagtgaaggaaaataacgcatcatgactattaatgtctccgaactacttgccaaagtccccacgggtctactgattggtgattcctgggtggaagcatccgagggcggtactttcgatgtggaaaacccagcgacgggtgaaacaatcgcaacgctcgcgtctgctacttccgaggatgcactggctgctcttgatgctgcatgcgctgttcaggccgagtgggctaggacgccagcgcgcgagcgttctaatattttacgacgcggtttcgagctcgtcgcggaacgtgcagaagagttcgccaccctcatgaccttggaaatgggcaaacctttggctgaagctcgcggcgaagtcacctacggcaacgaattcctgcgctggttctctgaggaagcagtccgcctctacggccgctacggtgctaccccagaaggcaacctgcgcatgatgaccacccgcaaaccagttggcccctgcctgttgatcaccccatggaacttcccactagcaatggccacccgtaaggttgcacccgccatcgctgcaggttgtgtcatggtgctcaagccagctcgcctgaccccgctgacctcccagtattttgcccagaccatgcttgatgccggtcttccagcaggtgtcctcaatgtggtctccggtgcttccgcctctgcgatttccaacccgattatggaagacgatcgccttcgtaaagtctcattcaccggctccaccccagttggccagcagctgctcaaaaaggctgccgataaagttctgcgcacctccatggaactcggcggcaacgcacctttcattgtcttcgaggacgccgacctagatctcgcgatcgaaggtgccatgggcgcaaaaatgcgcaacatcggcgaagcttgcaccgcagccaaccgtttcctagtccacgaatccgtcgccgatgaattcggccgacgcttcgcagcccgcctcgaggaacaagtcctaggcaacggcctcgacgaaggcgtcaccgtaggcccattggttgaggaaaaagcacgaaacagcgttgcatcgcttgtcgacgccgccgtctccgaaggtgccaccgtcctcaccggtggcaaggccggcacaggtgcaggctacttctacgaaccaacggtgctcacgggagtttcaacagatgcagccatcctgaacgaagagatcttcggtcccgtcgcaccgatcgtcaccttctctgatgaagctgaagctctgcgcctagccaattccaccgaatacggcctggcctcctacgtgttcacccaagacacctcacgcatcttccgcgtctccgacggcctcgagttcggcctagtgggcgtcaactccggtgtcatctctaacgccgctgcaccttttggtggcgtaaaacaatccggaatgggccgcgaaggtggtctcgaaggaattgaagagtacacctccgtgcagtacatcggtatccgggatccttacgccggctaggttttggcggatgagagaagattttcagcctgat

SEQ ID NO: 43 - DNA, 1807 bp, Artificial Sequence
  Synthesized
gcttgcatgcctgcaggtcgactctagaggatccccgtagtgctcgtcgtggtaggtgcgcagcagagattcaggcgcacgaccagaaagcacgtggctgagcttccagccggacgttgtggccggagtaaaaatccatccaaactttccgcgatgctggtaaacctgtggatgtcaatgcctttgatttgaactaagcacaggactacctcgacgccggcgccaactttgtccgagtcggtgccgatgtccagcaactcaacgctgctggatacgaaaagtgaaggaaaataacgcatcatgactattaatgtctccgaactacttgccaaagtccccacgggtctactgattggtgattcctgggtggaagcatccgagggcggtactttcgatgtggaaaacccagcgacgggtgaaacaatcgcaacgctcgcgtctgctacttccgaggatgcactggctgctcttgatgctgcatgcgctgttcaggccgagtgggctaggacgccagcgcgcgagcgttctaatattttacgacgcggtttcgagctcgtcgcggaacgtgcagaagagttcgccaccctcatgaccttggaaatgggcaaacctttggctgaagctcgcggcgaagtcacctacggcaacgaattcctgcgctggttctctgaggaagcagtccgcctctacggccgctacggtgctaccccagaaggcaacctgcgcatgatgaccacccgcaaaccagttggcccctgcctgttgatcaccccatggaacttcccactagcaatggccacccgtaaggttgcacccgccatcgctgcaggttgtgtcatggtgctcaagccagctcgcctgaccccgctgacctcccagtattttgcccagaccatacttgatgccggtcttccagcaggtgtcctcaatgtggtctccggtgcttccgcctctgcgatttccaacccgattatggaagacgatcgccttcgtaaagtctcattcaccggctccaccccagttggccagcagctgctcaaaaaggctgccgataaagttctgcgcacctccatggaactcggcggcaacgcacctttcattgtcttcgaggacgccgacctagatctcgcgatcgaaggtgccatgggcgcaaaaatgcgcaacatcggcgaagcttgcaccgcagccaaccgtttcctagtccacgaatccgtcgccgatgaattcggccgacgcttcgcagcccgcctcgaggaacaagtcctaggcaacggcctcgacgaaggcgtcaccgtaggcccattggttgaggaaaaagcacgaaacagcgttgcatcgcttgtcgacgccgccgtctccgaaggtgccaccgtcctcaccggtggcaaggccggcacaggtgcaggctacttctacgaaccaacggtgctcacgggagtttcaacagatgcagccatcctgaacgaagagatcttcggtcccgtcgcaccgatcgtcaccttctctgatgaagctgaagctctgcgcctagccaattccaccgaatacggcctggcctcctacgtgttcacccaagacacctcacgcatcttccgcgtctccgacggcctcgagttcggcctagtgggcgtcaactccggtgtcatctctaacgccgctgcaccttttggtggcgtaaaacaatccggaatgggccgcgaaggtggtctcgaaggaattgaagagtacacctccgtgcagtacatcggtatccgggatccttacgccggctaggttttggcggatgagagaagattttcagcctgat

SEQ ID NO: 44 - DNA, 1846 bp, Artificial Sequence
  Synthesized
agcggataacaatttcacacaggaaacagaattaattaagcttgcatgcctgcaggtcgactctagaggatccccgtagtgctcgtcgtggtaggtgcgcagcagagattcaggcgcacgaccagaaagcacgtggctgagcttccagccggacgttgtggccggagtaaaaatccatccaaactttccgcgatgctggtaaacctgtggatgtcaatgcctttgatttgaactaagcacaggactacctcgacgccggcgccaactttgtccgagtcggtgccgatgtccagcaactcaacgctgctggatacgaaaagtgaaggaaaataacgcatcatgactattaatgtctccgaactacttgccaaagtccccacgggtctactgattggtgattcctgggtggaagcatccgagggcggtactttcgatgtggaaaacccagcgacgggtgaaacaatcgcaacgctcgcgtctgctacttccgaggatgcactggctgctcttgatgctgcatgcgctgttcaggccgagtgggctaggacgccagcgcgcgagcgttctaatattttacgacgcggtttcgagctcgtcgcggaacgtgcagaagagttcgccaccctcatgaccttggaaatgggcaaacctttggctgaagctcgcggcgaagtcacctacggcaacgaattcctgcgctggttctctgaggaagcagtccgcctctacggccgctacggtgctaccccagaaggcaacctgcgcatgatgaccacccgcaaaccagttggcccctgcctgttgatcaccccatggaacttcccactagcaatggccacccgtaaggttgcacccgccatcgctgcaggttgtgtcatggtgctcaagccagctcgcctgaccccgctgacctcccagtattttgcccagaccatacttgatgccggtcttccagcaggtgtcctcaatgtggtctccggtgcttccgcctctgcgatttccaacccgattatggaagacgatcgccttcgtaaagtctcattcaccggctccaccccagttggccagcagctgctcaaaaaggctgccgataaagttctgcgcacctccatggaactcggcggcaacgcacctttcattgtcttcgaggacgccgacctagatctcgcgatcgaaggtgccatgggcgcaaaaatgcgcaacatcggcgaagcttgcaccgcagccaaccgtttcctagtccacgaatccgtcgccgatgaattcggccgacgcttcgcagcccgcctcgaggaacaagtcctaggcaacggcctcgacgaaggcgtcaccgtaggcccattggttgaggaaaaagcacgaaacagcgttgcatcgcttgtcgacgccgccgtctccgaaggtgccaccgtcctcaccggtggcaaggccggcacaggtgcaggctacttctacgaaccaacggtgctcacgggagtttcaacagatgcagccatcctgaacgaagagatcttcggtcccgtcgcaccgatcgtcaccttctctgatgaagctgaagctctgcgcctagccaattccaccgaatacggcctggcctcctacgtgttcacccaagacacctcacgcatcttccgcgtctccgacggcctcgagttcggcctagtgggcgtcaactccggtgtcatctctaacgccgctgcaccttttggtggcgtaaaacaatccggaatgggccgcgaaggtggtctcgaaggaattgaagagtacacctccgtgcagtacatcggtatccgggatccttacgccggctaggttttggcggatgagagaagattttcagcctgat

SEQ ID NO: 45 - DNA, 709 bp, Artificial Sequence
  Synthesized
cagtgccaagcttgcatgcctgcaggtcgactctaggtctgggggtgagcgcggatctgaggcggtgacgtattaccagtattcctggggtcgggcgcgtcgtagtttacgaggaatggaggagcagattgcaaaagctgagcgtgcggtagccggcctcgttccggtcaagcgttatcggtatgttgatcttaaagctgcacaaaagcaggtcaaccatgcattagcagataagtatcgggcgttggctggggtgaaaggatacgagacctcacgcagtgatcttgctgctggtgaggttattggggcatatcgtcagttgtttaaaattgagaaggcgtttcggatggcgaagtcggatttgaaggcttgtccgatttttcatcggaagaaggattcgattgatgcgcatttaacgattgtgatggtatcgatggctgtggggcatgtgttggaacagcggtcggggttgtcgttgaagcggttggtgcggatattgaagagataccgcactttcactgtggaggtggctggccacagggttttcgctcaggctccggttcctgatgatgttgcgttaattgttgatcggttacctaaaccgtcagactaaaatggcctaagtcaggcaaaacacaaaaaatccaccacaaacatcccagtgtttgcggtggatttgtaaaggggcagatggatgcgttattttcct

SEQ ID NO: 46 - DNA, 734 bp, Artificial Sequence
  Synthesized
tggatttgtaaaggggcagatggatgcgttattttccttcacttttcgtatccagcagcgttgagttgctggacatcggcaccgactcggacaaagttggcgccggcgtcgaggtagtcctgtgcttagttcaaatcaaaggcattgacatccacaggtttaccagcatcgcggaaagtttggatggatttttactccggccacaacgtccggctggaagctcagccacgtgctttctggtcgtgcgcctgaatctctgctgcgcacctaccacgacgagcactacccagctgcggcaaacctcattgctttcgataagggatggtccaccctcatggtccctcagctggaagatccagaggctgtggagaggtactacgttgctgcggaggaattcaccgccggattcctcaccgaaaaccaggacaatctgatcactgcgggcacggagcaccaggcgctcgcgagcggcttcccggtggggcgtcgcttcaagtccgatattgctttacgacgctgcgatgcggtgaccacccacatcggccacgaacactccgccgatggtcgatggaagaaagcgaagactcaccactcaaccgcttcaccccagaagacggcgaccgcaacgcagtcttcgatatcaaggccatctaccagcagcattaccactccttcgacctgttcgatgcgccagaggggtaccgagctcgaattcgtaatcatggtcatagctg

SEQ ID NO: 47 - DNA, 1405 bp, Artificial Sequence
  Synthesized
cagtgccaagcttgcatgcctgcaggtcgactctaggtctgggggtgagcgcggatctgaggcggtgacgtattaccagtattcctggggtcgggcgcgtcgtagtttacgaggaatggaggagcagattgcaaaagctgagcgtgcggtagccggcctcgttccggtcaagcgttatcggtatgttgatcttaaagctgcacaaaagcaggtcaaccatgcattagcagataagtatcgggcgttggctggggtgaaaggatacgagacctcacgcagtgatcttgctgctggtgaggttattggggcatatcgtcagttgtttaaaattgagaaggcgtttcggatggcgaagtcggatttgaaggcttgtccgatttttcatcggaagaaggattcgattgatgcgcatttaacgattgtgatggtatcgatggctgtggggcatgtgttggaacagcggtcggggttgtcgttgaagcggttggtgcggatattgaagagataccgcactttcactgtggaggtggctggccacagggttttcgctcaggctccggttcctgatgatgttgcgttaattgttgatcggttacctaaaccgtcagactaaaatggcctaagtcaggcaaaacacaaaaaatccaccacaaacatcccagtgtttgcggtggatttgtaaaggggcagatggatgcgttattttccttcacttttcgtatccagcagcgttgagttgctggacatcggcaccgactcggacaaagttggcgccggcgtcgaggtagtcctgtgcttagttcaaatcaaaggcattgacatccacaggtttaccagcatcgcggaaagtttggatggatttttactccggccacaacgtccggctggaagctcagccacgtgctttctggtcgtgcgcctgaatctctgctgcgcacctaccacgacgagcactacccagctgcggcaaacctcattgctttcgataagggatggtccaccctcatggtccctcagctggaagatccagaggctgtggagaggtactacgttgctgcggaggaattcaccgccggattcctcaccgaaaaccaggacaatctgatcactgcgggcacggagcaccaggcgctcgcgagcggcttcccggtggggcgtcgcttcaagtccgatattgctttacgacgctgcgatgcggtgaccacccacatcggccacgaacactccgccgatggtcgatggaagaaagcgaagactcaccactcaaccgcttcaccccagaagacggcgaccgcaacgcagtcttcgatatcaaggccatctaccagcagcattaccactccttcgacctgttcgatgcgccagaggggtaccgagctcgaattcgtaatcatggtcatagctg

SEQ ID NO: 48 - DNA, 2804 bp, Artificial Sequence
  Synthesized
gtctgggggtgagcgcggatctgaggcggtgacgtattaccagtattcctggggtcgggcgcgtcgtagtttacgaggaatggaggagcagattgcaaaagctgagcgtgcggtagccggcctcgttccggtcaagcgttatcggtatgttgatcttaaagctgcacaaaagcaggtcaaccatgcattagcagataagtatcgggcgttggctggggtgaaaggatacgagacctcacgcagtgatcttgctgctggtgaggttattggggcatatcgtcagttgtttaaaattgagaaggcgtttcggatggcgaagtcggatttgaaggcttgtccgatttttcatcggaagaaggattcgattgatgcgcatttaacgattgtgatggtatcgatggctgtggggcatgtgttggaacagcggtcggggttgtcgttgaagcggttggtgcggatattgaagagataccgcactttcactgtggaggtggctggccacagggttttcgctcaggctccggttcctgatgatgttgcgttaattgttgatcggttacctaaaccgtcagactaaaatggcctaagtcaggcaaaacacaaaaaatccaccacaaacatcccagtgtttgcggtggatttgtaaaggggcagatgctagccggcgtaaggatcccggataccgatgtactgcacggaggtgtactcttcaattccttcgagaccaccttcgcggcccattccggattgttttacgccaccaaaaggtgcagcggcgttagagatgacaccggagttgacgcccactaggccgaactcgaggccgtcggagacgcggaagatgcgtgaggtgtcttgggtgaacacgtaggaggccaggccgtattcggtggaattggctaggcgcagagcttcagcttcatcagagaaggtgacgatcggtgcgacgggaccgaagatctcttcgttcaggatggctgcatctgttgaaactcccgtgagcaccgttggttcgtagaagtagcctgcacctgtgccggccttgccaccggtgaggacggtggcaccttcggagacggcggcgtcgacaagcgatgcaacgctgtttcgtgctttttcctcaaccaatgggcctacggtgacgccttcgtcgaggccgttgcctaggacttgttcctcgaggcgggctgcgaagcgtcggccgaattcatcggcgacggattcgtggactaggaaacggttggctgcggtgcaagcttcgccgatgttgcgcatttttgcgcccatggcaccttcgatcgcgagatctaggtcggcgtcctcgaagacaatgaaaggtgcgttgccgccgagttccatggaggtgcgcagaactttatcggcagcctttttgagcagctgctggccaactggggtggagccggtgaatgagactttacgaaggcgatcgtcttccataatcgggttggaaatcgcagaggcggaagcaccggagaccacattgaggacacctgctggaagaccggcatcaagcatggtctgggcaaaatactgggaggtcagcggggtcaggcgagctggcttgagcaccatgacacaacctgcagcgatggcgggtgcaaccttacgggtggccattgctagtgggaagttccatggggtgatcaacaggcaggggccaactggtttgcgggtggtcatcatgcgcaggttgccttctggggtagcaccgtagcggccgtagaggcggactgcttcctcagagaaccagcgcaggaattcgttgccgtaggtgacttcgccgcgagcttcagccaaaggtttgcccatttccaaggtcatgagggtggcgaactcttctgcacgttccgcgacgagctcgaaaccgcgtcgtaaaatattagaacgctcgcgcgctggcgtcctagcccactcggcctgaacagcgcatgcagcatcaagagcagccagtgcatcctcggaagtagcagacgcgagcgttgcgattgtttcacccgtcgctgggttttccacatcgaaagtaccgccctcggatgcttccacccaggaatcaccaatcagtagacccgtggggactttggcaagtagttcggagacattaatagtcatgatgcgttattttccttcacttttcgtatccagcagcgttgagttgctggacatcggcaccgactcggacaaagttggcgccggcgtcgaggtagtcctgtgcttagttcaaatcaaaggcattgacatccacaggtttaccagcatcgcggaaagtttggatggatttttactccggccacaacgtccggctggaagctcagccacgtgctttctggtcgtgcgcctgaatctctgctgcgcacctaccacgacgagcactacccagctgcggcaaacctcattgctttcgataagggatggtccaccctcatggtccctcagctggaagatccagaggctgtggagaggtactacgttgctgcggaggaattcaccgccggattcctcaccgaaaaccaggacaatctgatcactgcgggcacggagcaccaggcgctcgcgagcggcttcccggtggggcgtcgcttcaagtccgatattgctttacgacgctgcgatgcggtgaccacccacatcggccacgaacactccgccgatggtcgatggaagaaagcgaagactcaccactcaaccgcttcaccccagaagacggcgaccgcaacgcagtcttcgatatcaaggccatctaccagcagcattaccactccttcgacctgttcgatgcgccagac

SEQ ID NO: 49 - DNA, 1331 bp, Artificial Sequence
  Synthesized
gtctgggggtgagcgcggatctgaggcggtgacgtattaccagtattcctggggtcgggcgcgtcgtagtttacgaggaatggaggagcagattgcaaaagctgagcgtgcggtagccggcctcgttccggtcaagcgttatcggtatgttgatcttaaagctgcacaaaagcaggtcaaccatgcattagcagataagtatcgggcgttggctggggtgaaaggatacgagacctcacgcagtgatcttgctgctggtgaggttattggggcatatcgtcagttgtttaaaattgagaaggcgtttcggatggcgaagtcggatttgaaggcttgtccgatttttcatcggaagaaggattcgattgatgcgcatttaacgattgtgatggtatcgatggctgtggggcatgtgttggaacagcggtcggggttgtcgttgaagcggttggtgcggatattgaagagataccgcactttcactgtggaggtggctggccacagggttttcgctcaggctccggttcctgatgatgttgcgttaattgttgatcggttacctaaaccgtcagactaaaatggcctaagtcaggcaaaacacaaaaaatccaccacaaacatcccagtgtttgcggtggatttgtaaaggggcagatggatgcgttattttccttcacttttcgtatccagcagcgttgagttgctggacatcggcaccgactcggacaaagttggcgccggcgtcgaggtagtcctgtgcttagttcaaatcaaaggcattgacatccacaggtttaccagcatcgcggaaagtttggatggatttttactccggccacaacgtccggctggaagctcagccacgtgctttctggtcgtgcgcctgaatctctgctgcgcacctaccacgacgagcactacccagctgcggcaaacctcattgctttcgataagggatggtccaccctcatggtccctcagctggaagatccagaggctgtggagaggtactacgttgctgcggaggaattcaccgccggattcctcaccgaaaaccaggacaatctgatcactgcgggcacggagcaccaggcgctcgcgagcggcttcccggtggggcgtcgcttcaagtccgatattgctttacgacgctgcgatgcggtgaccacccacatcggccacgaacactccgccgatggtcgatggaagaaagcgaagactcaccactcaaccgcttcaccccagaagacggcgaccgcaacgcagtcttcgatatcaaggccatctaccagcagcattaccactccttcgacctgttcgatgcgccagag